European Patent Specification EP 3 350 215 B1, published December 3, 2025. Title: CYSTINE KNOT SCAFFOLD PLATFORM. Applicant: Genentech, Inc. The sequence listing filed with the application follows.

SEQUENCE LISTING (568 sequences)

SEQ ID NO: 1 - protein, 28 aa, Ecballium elaterium
GCPRILMRCKQDSDCLAGCVCGPNGFCG

SEQ ID NO: 2 - protein, 6 aa, Artificial Sequence
  Synthetic Construct
  VARIANT 1, 2, 3, 4, 5, 6: Xaa = Any Amino Acid
XXXXXX

SEQ ID NO: 3 - protein, 7 aa, Artificial Sequence
  Synthetic Construct
  VARIANT 1, 2, 3, 4, 5, 6, 7: Xaa = Any Amino Acid
XXXXXXX

SEQ ID NO: 4 - protein, 8 aa, Artificial Sequence
  Synthetic Construct
  VARIANT 1, 2, 3, 4, 5, 6, 7, 8: Xaa = Any Amino Acid
XXXXXXXX

SEQ ID NO: 5 - protein, 9 aa, Artificial Sequence
  Synthetic Construct
  VARIANT 1, 2, 3, 4, 5, 6, 7, 8, 9: Xaa = Any Amino Acid
XXXXXXXXX

SEQ ID NO: 6 - protein, 10 aa, Artificial Sequence
  Synthetic Construct
  VARIANT 1, 2, 3, 4, 5, 6, 7, 8, 9, 10: Xaa = Any Amino Acid
XXXXXXXXXX

SEQ ID NO: 7 - protein, 5 aa, Artificial Sequence
  Synthetic Construct
  VARIANT 1, 2, 3, 4, 5: Xaa = any amino acid or an unnatural amino acid
XXXXX

SEQ ID NO: 8 - protein, 8 aa, Artificial Sequence
  Synthetic Construct
PTTRFKQY

SEQ ID NO: 9 - protein, 10 aa, Artificial Sequence
  Synthetic Construct
QDPTFNWALY

SEQ ID NO: 10 - protein, 8 aa, Artificial Sequence
  Synthetic Construct
QLMQPFWG

SEQ ID NO: 11 - protein, 8 aa, Artificial Sequence
  Synthetic Construct
RDLDVKWD

SEQ ID NO: 12 - protein, 10 aa, Artificial Sequence
  Synthetic Construct
RTPWEPHDIT

SEQ ID NO: 13 - protein, 10 aa, Artificial Sequence
  Synthetic Construct
TTPWPPHEIM

SEQ ID NO: 14 - protein, 10 aa, Artificial Sequence
  Synthetic Construct
VTPWKPHWIN

SEQ ID NO: 15 - protein, 5 aa, Artificial Sequence
  Synthetic Construct
GPNGF

SEQ ID NO: 16 - protein, 5 aa, Artificial Sequence
  Synthetic Construct
QMYQS

SEQ ID NO: 17 - protein, 5 aa, Artificial Sequence
  Synthetic Construct
HWYQS

SEQ ID NO: 18 - protein, 5 aa, Artificial Sequence
  Synthetic Construct
QYYSS

SEQ ID NO: 19 - protein, 5 aa, Artificial Sequence
  Synthetic Construct
GPNGF

SEQ ID NO: 20 - protein, 5 aa, Artificial Sequence
  Synthetic Construct
  VARIANT 1: Xaa = G or E or Y or Q or H
  VARIANT 2: Xaa = P or M or W or Y
  VARIANT 3: Xaa = N or Y or W
  VARIANT 4: Xaa = G or D or T or Q or R or S
  VARIANT 5: Xaa = F or A or E or S
XXXXX

SEQ ID NO: 21 - protein, 30 aa, Artificial Sequence
  Synthetic Construct
GCPTTRFKQYCKQDSDCLAGCVCGPNGFCG

SEQ ID NO: 22 - protein, 32 aa, Artificial Sequence
  Synthetic Construct
GCQDPTFNWALYCKQDSDCLAGCVCQMYQSCG

SEQ ID NO: 23 - protein, 30 aa, Artificial Sequence
  Synthetic Construct
GCQLMQPFWGCKQDSDCLAGCVCHWYQSCG

SEQ ID NO: 24 - protein, 30 aa, Artificial Sequence
  Synthetic Construct
GCRDLDVKWDCKQDSDCLAGCFCQYYSSCG

SEQ ID NO: 25 - protein, 32 aa, Artificial Sequence
  Synthetic Construct
GCRTPWEPHDITCKQDSDCLAGCVCGPNGFCG

SEQ ID NO: 26 - protein, 32 aa, Artificial Sequence
  Synthetic Construct
GCTTPWPPHEIMCKQDSDCLAGCVCGPNGFCG

SEQ ID NO: 27 - protein, 32 aa, Artificial Sequence
  Synthetic Construct
GCVTPWKPHWINCKQDSDCLAGCVCGPNGFCG

SEQ ID NO: 28 - protein, 8 aa, Artificial Sequence
  Synthetic Construct
DVLQPFWG

SEQ ID NO: 29 - protein, 8 aa, Artificial Sequence
  Synthetic Construct
QISQPFWG

SEQ ID NO: 30 - protein, 8 aa, Artificial Sequence
  Synthetic Construct
DRMQPLWG

SEQ ID NO: 31 - protein, 8 aa, Artificial Sequence
  Synthetic Construct
NLMLPFWG

SEQ ID NO: 32 - protein, 8 aa, Artificial Sequence
  Synthetic Construct
QRTQPFWG

SEQ ID NO: 33 - protein, 8 aa, Artificial Sequence
  Synthetic Construct
NIMLPFWG

SEQ ID NO: 34 - protein, 8 aa, Artificial Sequence
  Synthetic Construct
DPMQPFWG

SEQ ID NO: 35 - protein, 8 aa, Artificial Sequence
  Synthetic Construct
DVMQPYWG

SEQ ID NO: 36 - protein, 8 aa, Artificial Sequence
  Synthetic Construct
DIMQPLWG

SEQ ID NO: 37 - protein, 8 aa, Artificial Sequence
  Synthetic Construct
QLLQPLWG

SEQ ID NO: 38 - protein, 8 aa, Artificial Sequence
  Synthetic Construct
NPMLPLWG

SEQ ID NO: 39 - protein, 8 aa, Artificial Sequence
  Synthetic Construct
KLFEPLWG

SEQ ID NO: 40 - protein, 8 aa, Artificial Sequence
  Synthetic Construct
  VARIANT 1: Xaa = Q or D or K or N or A or R or H
  VARIANT 2: Xaa = L or V or I or R or P or V
  VARIANT 3: Xaa = M or L or S or T or F
  VARIANT 4: Xaa = Q or E or L or H
  VARIANT 6: Xaa = F or L or M or Y or S
XXXXPXWG

SEQ ID NO: 41 - protein, 5 aa, Artificial Sequence
  Synthetic Construct
HFYNS

SEQ ID NO: 42 - protein, 5 aa, Artificial Sequence
  Synthetic Construct
LWYKS

SEQ ID NO: 43 - protein, 5 aa, Artificial Sequence
  Synthetic Construct
RWYHS

SEQ ID NO: 44 - protein, 5 aa, Artificial Sequence
  Synthetic Construct
RWYQS

SEQ ID NO: 45 - protein, 5 aa, Artificial Sequence
  Synthetic Construct
QYYQS

SEQ ID NO: 46 - protein, 5 aa, Artificial Sequence
  Synthetic Construct
HWYNS

SEQ ID NO: 47 - protein, 30 aa, Artificial Sequence
  Synthetic Construct
GCDVLQPFWGCKQDSDCLAGCVCHWYQSCG

SEQ ID NO: 48 - protein, 30 aa, Artificial Sequence
  Synthetic Construct
GCQISQPFWGCKQDSDCLAGCVCHFYNSCG

SEQ ID NO: 49 - protein, 30 aa, Artificial Sequence
  Synthetic Construct
GCDRMQPLWGCKQDSDCLAGCVCLWYKSCG

SEQ ID NO: 50 - protein, 30 aa, Artificial Sequence
  Synthetic Construct
GCNLMLPFWGCKQDSDCLAGCVCRWYHSCG

SEQ ID NO: 51 - protein, 30 aa, Artificial Sequence
  Synthetic Construct
GCQRTQPFWGCKQDSDCLAGCVCRWYQSCG

SEQ ID NO: 52 - protein, 30 aa, Artificial Sequence
  Synthetic Construct
GCNIMLPFWGCKQDSDCLAGCVCQYYQSCG

SEQ ID NO: 53 - protein, 30 aa, Artificial Sequence
  Synthetic Construct
GCNPMLPFWGCKQDSDCLAGCVCHWYQSCG

SEQ ID NO: 54 - protein, 30 aa, Artificial Sequence
  Synthetic Construct
GCDPMQPFWGCKQDSDCLAGCVCRWYQSCG

SEQ ID NO: 55 - protein, 30 aa, Artificial Sequence
  Synthetic Construct
GCDVMQPYWGCKQDSDCLAGCVCHWYNSCG

SEQ ID NO: 56 - protein, 30 aa, Artificial Sequence
  Synthetic Construct
GCDIMQPLWGCKQDSDCLAGCVCHWYQSCG

SEQ ID NO: 57 - protein, 30 aa, Artificial Sequence
  Synthetic Construct
GCQLLQPLWGCKQDSDCLAGCVCRWYQSCG

SEQ ID NO: 58 - protein, 30 aa, Artificial Sequence
  Synthetic Construct
GCNPMLPLWGCKQDSDCLAGCVCHWYQSCG

SEQ ID NO: 59 - protein, 30 aa, Artificial Sequence
  Synthetic Construct
GCKLFEPLWGCKQDSDCLAGCVCRWYESCG

SEQ ID NO: 60 - protein, 10 aa, Artificial Sequence
  Synthetic Construct
KNPLFNWALY

SEQ ID NO: 61 - protein, 10 aa, Artificial Sequence
  Synthetic Construct
QDPTVNWAVY

SEQ ID NO: 62 - protein, 10 aa, Artificial Sequence
  Synthetic Construct
QDPTFNWAEY

SEQ ID NO: 63 - protein, 10 aa, Artificial Sequence
  Synthetic Construct
QDPSLNWADY

SEQ ID NO: 64 - protein, 10 aa, Artificial Sequence
  Synthetic Construct
LDRTLNWALY

SEQ ID NO: 65 - protein, 10 aa, Artificial Sequence
  Synthetic Construct
LDPSFNWSLY

SEQ ID NO: 66 - protein, 10 aa, Artificial Sequence
  Synthetic Construct
RDLTINWALF

SEQ ID NO: 67 - protein, 10 aa, Artificial Sequence
  Synthetic Construct
LDPTVNWALF

SEQ ID NO: 68 - protein, 10 aa, Artificial Sequence
  Synthetic Construct
QDPKLNWAVY

SEQ ID NO: 69 - protein, 10 aa, Artificial Sequence
  Synthetic Construct
LDPSFDWALY

SEQ ID NO: 70 - protein, 10 aa, Artificial Sequence
  Synthetic Construct
  VARIANT 1: Xaa = Q or D or K or W or E or L or R
  VARIANT 2: Xaa = D or N
  VARIANT 3: Xaa = P or R or L or T
  VARIANT 4: Xaa = T or S or L or K
  VARIANT 5: Xaa = F or V or L or I
  VARIANT 6: Xaa = N or D
  VARIANT 8: Xaa = A or S or G
  VARIANT 9: Xaa = L or V or E or T or Q or D
  VARIANT 10: Xaa = F or Y
XXXXXXWXXX

SEQ ID NO: 71 - protein, 5 aa, Artificial Sequence
  Synthetic Construct
QLFDS

SEQ ID NO: 72 - protein, 5 aa, Artificial Sequence
  Synthetic Construct
QFYQS

SEQ ID NO: 73 - protein, 5 aa, Artificial Sequence
  Synthetic Construct
QLYQS

SEQ ID NO: 74 - protein, 5 aa, Artificial Sequence
  Synthetic Construct
QMHQS

SEQ ID NO: 75 - protein, 5 aa, Artificial Sequence
  Synthetic Construct
QMYNS

SEQ ID NO: 76 - protein, 5 aa, Artificial Sequence
  Synthetic Construct
QMYDS

SEQ ID NO: 77 - protein, 5 aa, Artificial Sequence
  Synthetic Construct
QHYKT

SEQ ID NO: 78 - protein, 5 aa, Artificial Sequence
  Synthetic Construct
QLFNS

SEQ ID NO: 79 - protein, 5 aa, Artificial Sequence
  Synthetic Construct
QLYNS

SEQ ID NO: 80 - protein, 5 aa, Artificial Sequence
  Synthetic Construct
  VARIANT 1: Xaa = Q or R
  VARIANT 2: Xaa = M or L or F or H
  VARIANT 3: Xaa = Y or F or H
  VARIANT 4: Xaa = D or Q or N or K
  VARIANT 5: Xaa = S or T
XXXXX

SEQ ID NO: 81 - protein, 32 aa, Artificial Sequence
  Synthetic Construct
GCKNPLFNWALYCKQDSDCLAGCVCQLFDSCG

SEQ ID NO: 82 - protein, 32 aa, Artificial Sequence
  Synthetic Construct
GCQDPTVNWAVYCKQDSDCLAGCVCQFYQSCG

SEQ ID NO: 83 - protein, 32 aa, Artificial Sequence
  Synthetic Construct
GCQDPTFNWAEYCKQDSDCLAGCVCQLYQSCG

SEQ ID NO: 84 - protein, 32 aa, Artificial Sequence
  Synthetic Construct
GCQDPTFNWAEYCKQDSDCLAGCVCQMYQSCG

SEQ ID NO: 85 - protein, 32 aa, Artificial Sequence
  Synthetic Construct
GCQDPSLNWADYCKQDSDCLAGCVCQMHQSCG

SEQ ID NO: 86 - protein, 32 aa, Artificial Sequence
  Synthetic Construct
GCLDRTLNWALYCKQDSDCLAGCVCQMYNSCG

SEQ ID NO: 87 - protein, 32 aa, Artificial Sequence
  Synthetic Construct
GCLDPSFNWSLYCKQDSDCLAGCVCQMYDSCG

SEQ ID NO: 88 - protein, 32 aa, Artificial Sequence
  Synthetic Construct
GCRDLTINWALFCKQDSDCLAGCVCQMFNSCG

SEQ ID NO: 89 - protein, 32 aa, Artificial Sequence
  Synthetic Construct
GCLDPTVNWALFCKQDSDCLAGCVCQHYKTCG

SEQ ID NO: 90 - protein, 32 aa, Artificial Sequence
  Synthetic Construct
GCQDPKLNWAVYCKQDSDCLAGCVCQLFNSCG

SEQ ID NO: 91 - protein, 32 aa, Artificial Sequence
  Synthetic Construct
GCLDPSFDWALYCKQDSDCLAGCVCQLYNSCG

SEQ ID NO: 92 - protein, 6 aa, Artificial Sequence
  Synthetic Construct
PRILMR

SEQ ID NO: 93 - protein, 5 aa, Artificial Sequence
  Synthetic Construct
KQDSD

SEQ ID NO: 94 - protein, 5 aa, Artificial Sequence
  Synthetic Construct
GQSFE

SEQ ID NO: 95 - protein, 5 aa, Artificial Sequence
  Synthetic Construct
GLDYD

SEQ ID NO: 96 - protein, 5 aa, Artificial Sequence
  Synthetic Construct
GPDLQ

SEQ ID NO: 97 - protein, 5 aa, Artificial Sequence
  Synthetic Construct
GRDFE

SEQ ID NO: 98 - protein, 5 aa, Artificial Sequence
  Synthetic Construct
  VARIANT 1: Xaa = K or G or Q or S or N
  VARIANT 2: Xaa = Q or L or P or A or V or T or R or W or K or G or Y
  VARIANT 3: Xaa = D or S or E or N
  VARIANT 4: Xaa = S or F or Y or L or F or Q or M
  VARIANT 5: Xaa = D or E or N or A or L or F or H or Q
XXXXX

SEQ ID NO: 99 - protein, 30 aa, Artificial Sequence
  Synthetic Construct
GCNIMLPFWGCGQSFECLAGCVCQYYQSCG

SEQ ID NO: 100 - protein, 30 aa, Artificial Sequence
  Synthetic Construct
GCNIMLPFWGCGLDYDCLAGCVCQYYQSCG

SEQ ID NO: 101 - protein, 30 aa, Artificial Sequence
  Synthetic Construct
GCNIMLPFWGCGPDLQCLAGCVCQYYQSCG

SEQ ID NO: 102 - protein, 30 aa, Artificial Sequence
  Synthetic Construct
GCNIMLPFWGCGRDFECLAGCVCQYYQSCG

SEQ ID NO: 103 - protein, 30 aa, Artificial Sequence
  Synthetic Construct
GCNIMLPFWGCGRDFECLQQCICQYYQSCG

SEQ ID NO: 104 - protein, 30 aa, Artificial Sequence
  Synthetic Construct
GCNIMLPFWGCGRDFECVERCICQYYQSCG

SEQ ID NO: 105 - protein, 30 aa, Artificial Sequence
  Synthetic Construct
GCNIMLPFWGCGRDFECMSDCICQYYQSCG

SEQ ID NO: 106 - protein, 30 aa, Artificial Sequence
  Synthetic Construct
GCNIMLPFWGCGRDFECMNQCICQYYQSCG

SEQ ID NO: 107 - protein, 30 aa, Artificial Sequence
  Synthetic Construct
GCNIMLPFWGCGRDFECMQTCICQYYQSCG

SEQ ID NO: 108 - protein, 30 aa, Artificial Sequence
  Synthetic Construct
GCNIMLPFWGCGRDFECVYQCICQYYQSCG

SEQ ID NO: 109 - protein, 30 aa, Artificial Sequence
  Synthetic Construct
GCNIMLPFWGCGRDFECFINCICQYYQSCG

SEQ ID NO: 110 - protein, 30 aa, Artificial Sequence
  Synthetic Construct
GCNIMLPFWGCGRDFECVSQCICQYYQSCG

SEQ ID NO: 111 - protein, 30 aa, Artificial Sequence
  Synthetic Construct
GCNIMLPFWGCGRDFECVTECICQYYQSCG

SEQ ID NO: 112 - protein, 30 aa, Artificial Sequence
  Synthetic Construct
GCNIMLPFWGCGRDFECFYECICQYYQSCG

SEQ ID NO: 113 - protein, 30 aa, Artificial Sequence
  Synthetic Construct
GCNIMLPFWGCGRDFECMEQCICQYYQSCG

SEQ ID NO: 114 - protein, 30 aa, Artificial Sequence
  Synthetic Construct
GCNIMLPFWGCGRDFECVYRCICQYYQSCG

SEQ ID NO: 115 - protein, 8 aa, Artificial Sequence
  Synthetic Construct
  VARIANT 1: Xaa = K or P or Q or R
  VARIANT 2: Xaa = K or T or L or D
  VARIANT 3: Xaa = W or T or M or L
  VARIANT 4: Xaa = Q or R or D
  VARIANT 5: Xaa = W or F or P or V
  VARIANT 6: Xaa = W or K or F
  VARIANT 7: Xaa = Y or Q or W
  VARIANT 8: Xaa = M or Y or G or D
XXXXXXXX

SEQ ID NO: 116 - skipped

SEQ ID NO: 117 - protein, 5 aa, Artificial Sequence
  Synthetic Construct
GENFL

SEQ ID NO: 118 - protein, 5 aa, Artificial Sequence
  Synthetic Construct
GPDID

SEQ ID NO: 119 - protein, 5 aa, Artificial Sequence
  Synthetic Construct
GRDMD

SEQ ID NO: 120 - protein, 5 aa, Artificial Sequence
  Synthetic Construct
EMDFD

SEQ ID NO: 121 - protein, 5 aa, Artificial Sequence
  Synthetic Construct
  VARIANT 1: Xaa = K or G or D or A or E
  VARIANT 2: Xaa = Q or E or R or V or P or D or M or G or N or L or A or F
  VARIANT 3: Xaa = D or N or Y or S
  VARIANT 4: Xaa = S or F or L or I or M or Y or V or N or E
  VARIANT 5: Xaa = D or L or Q or S or E or T or L or A or N
XXXXX

SEQ ID NO: 122 - protein, 30 aa, Artificial Sequence
  Synthetic Construct
GCDVMQPYWGCGENFLCLAGCVCHWYNSCG

SEQ ID NO: 123 - protein, 30 aa, Artificial Sequence
  Synthetic Construct
GCDVMQPYWGCGPDIDCLAGCVCHWYNSCG

SEQ ID NO: 124 - protein, 30 aa, Artificial Sequence
  Synthetic Construct
GCDVMQPYWGCGRDMDCLAGCVCHWYNSCG

SEQ ID NO: 125 - protein, 30 aa, Artificial Sequence
  Synthetic Construct
GCDVMQPYWGCEMDFDCLAGCVCHWYNSCG

SEQ ID NO: 126 - protein, 30 aa, Artificial Sequence
  Synthetic Construct
GCDVMQPYWGCGESLSCLAGCVCHWYNSCG

SEQ ID NO: 127 - protein, 8 aa, Artificial Sequence
  Synthetic Construct
DVMKPMWG

SEQ ID NO: 128 - protein, 8 aa, Artificial Sequence
  Synthetic Construct
DVLDPTWG

SEQ ID NO: 129 - protein, 8 aa, Artificial Sequence
  Synthetic Construct
DVLQPLWG

SEQ ID NO: 130 - protein, 8 aa, Artificial Sequence
  Synthetic Construct
  VARIANT 3: Xaa = M or L
  VARIANT 4: Xaa = Q or K or D
  VARIANT 6: Xaa = Y or M or T or L
DVXXPXWG

SEQ ID NO: 131 - protein, 5 aa, Artificial Sequence
  Synthetic Construct
QWYNS

SEQ ID NO: 132 - protein, 5 aa, Artificial Sequence
  Synthetic Construct
LWYNS

SEQ ID NO: 133 - protein, 5 aa, Artificial Sequence
  Synthetic Construct
RWYNS

SEQ ID NO: 134 - protein, 5 aa, Artificial Sequence
  Synthetic Construct
  VARIANT 1: Xaa = H or L or Q or R
XWYNS

SEQ ID NO: 135 - protein, 30 aa, Artificial Sequence
  Synthetic Construct
GCDVMKPMWGCKQDSDCLAGCVCQWYNSCG

SEQ ID NO: 136 - protein, 30 aa, Artificial Sequence
  Synthetic Construct
GCDVLDPTWGCKQDSDCLAGCVCLWYNSCG

SEQ ID NO: 137 - protein, 30 aa, Artificial Sequence
  Synthetic Construct
GCDVLQPLWGCKQDSDCLAGCVCRWYNSCG

SEQ ID NO: 138 - skipped

SEQ ID NO: 139 - protein, 30 aa, Artificial Sequence
  Synthetic Construct
GCDVMQPYWGCGPDIDCFVRCLCHWYNSCG

SEQ ID NO: 140 - protein, 30 aa, Artificial Sequence
  Synthetic Construct
GCDVMQPYWGCGPDIDCLSNCICHWYNSCG

SEQ ID NO: 141 - protein, 8 aa, Artificial Sequence
  Synthetic Construct
NIMLPYWG

SEQ ID NO: 142 - protein, 30 aa, Artificial Sequence
  Synthetic Construct
GCNIMLPYWGCGRDFECMEQCICQYYQSCG

SEQ ID NO: 143 - protein, 8 aa, Artificial Sequence
  Synthetic Construct
  VARIANT 3: Xaa = norleucine
NIXLPYWG

SEQ ID NO: 144 - protein, 30 aa, Artificial Sequence
  Synthetic Construct
  VARIANT 5: Xaa = norleucine
GCNIXLPFWGCGRDFECMSDCICQYYQSCG

SEQ ID NO: 145 - protein, 30 aa, Artificial Sequence
  Synthetic Construct
  VARIANT 5: Xaa = norleucine
GCNIXLPFWGCGRDFECVSQCICQYYQSCG

SEQ ID NO: 146 - protein, 30 aa, Artificial Sequence
  Synthetic Construct
  VARIANT 5: Xaa = norleucine
GCNIXLPYWGCGRDFECMEQCICQYYQSCG

SEQ ID NO: 147 - protein, 8 aa, Artificial Sequence
  Synthetic Construct
RTNRVKGG

SEQ ID NO: 148 - protein, 6 aa, Artificial Sequence
  Synthetic Construct
VNRVRG

SEQ ID NO: 149 - protein, 8 aa, Artificial Sequence
  Synthetic Construct
MNHVKARR

SEQ ID NO: 150 - protein, 6 aa, Artificial Sequence
  Synthetic Construct
RSVNKI

SEQ ID NO: 151 - protein, 6 aa, Artificial Sequence
  Synthetic Construct
VNKIKG

SEQ ID NO: 152 - protein, 6 aa, Artificial Sequence
  Synthetic Construct
RNSIKR

SEQ ID NO: 153 - protein, 8 aa, Artificial Sequence
  Synthetic Construct
VSNRVNKG

SEQ ID NO: 154 - protein, 6 aa, Artificial Sequence
  Synthetic Construct
RGNIIK

SEQ ID NO: 155 - protein, 10 aa, Artificial Sequence
  Synthetic Construct
RSGNTIRKRE

SEQ ID NO: 156 - protein, 10 aa, Artificial Sequence
  Synthetic Construct
ASSNSIRQGW

SEQ ID NO: 157 - protein, 6 aa, Artificial Sequence
  Synthetic Construct
RSNRIR

SEQ ID NO: 158 - protein, 10 aa, Artificial Sequence
  Synthetic Construct
RSNKLREARG

SEQ ID NO: 159 - protein, 6 aa, Artificial Sequence
  Synthetic Construct
VNSVKR

SEQ ID NO: 160 - protein, 8 aa, Artificial Sequence
  Synthetic Construct
GSNKIRPR

SEQ ID NO: 161 - protein, 6 aa, Artificial Sequence
  Synthetic Construct
NRIRNS

SEQ ID NO: 162 - protein, 6 aa, Artificial Sequence
  Synthetic Construct
SRNSIK

SEQ ID NO: 163 - protein, 6 aa, Artificial Sequence
  Synthetic Construct
SNYVKR

SEQ ID NO: 164 - protein, 8 aa, Artificial Sequence
  Synthetic Construct
RANRVSGR

SEQ ID NO: 165 - protein, 8 aa, Artificial Sequence
  Synthetic Construct
SNRVKVRA

SEQ ID NO: 166 - protein, 6 aa, Artificial Sequence
  Synthetic Construct
ENRTKG

SEQ ID NO: 167 - protein, 6 aa, Artificial Sequence
  Synthetic Construct
GNKIRA

SEQ ID NO: 168 - protein, 8 aa, Artificial Sequence
  Synthetic Construct
ANRVKRTS

SEQ ID NO: 169 - protein, 5 aa, Artificial Sequence
  Synthetic Construct
SGGRD

SEQ ID NO: 170 - protein, 5 aa, Artificial Sequence
  Synthetic Construct
GSSRN

SEQ ID NO: 171 - protein, 5 aa, Artificial Sequence
  Synthetic Construct
GVEGR

SEQ ID NO: 172 - protein, 5 aa, Artificial Sequence
  Synthetic Construct
SVGHG

SEQ ID NO: 173 - protein, 5 aa, Artificial Sequence
  Synthetic Construct
NESRG

SEQ ID NO: 174 - protein, 5 aa, Artificial Sequence
  Synthetic Construct
GGPGG

SEQ ID NO: 175 - protein, 5 aa, Artificial Sequence
  Synthetic Construct
GPKSN

SEQ ID NO: 176 - protein, 5 aa, Artificial Sequence
  Synthetic Construct
YGHGD

SEQ ID NO: 177 - protein, 5 aa, Artificial Sequence
  Synthetic Construct
GSRQD

SEQ ID NO: 178 - protein, 5 aa, Artificial Sequence
  Synthetic Construct
SRGVN

SEQ ID NO: 179 - protein, 5 aa, Artificial Sequence
  Synthetic Construct
GPNDF

SEQ ID NO: 180 - protein, 5 aa, Artificial Sequence
  Synthetic Construct
GRGDY

SEQ ID NO: 181 - protein, 5 aa, Artificial Sequence
  Synthetic Construct
ASGSS

SEQ ID NO: 182 - protein, 5 aa, Artificial Sequence
  Synthetic Construct
SPGGR

SEQ ID NO: 183 - protein, 5 aa, Artificial Sequence
  Synthetic Construct
GFRGT

SEQ ID NO: 184 - protein, 5 aa, Artificial Sequence
  Synthetic Construct
RDRVG

SEQ ID NO: 185 - protein, 6 aa, Artificial Sequence
  Synthetic Construct
  VARIANT 1: Xaa = V or R or N or S or E or G
  VARIANT 2: Xaa = N or S or G or R
  VARIANT 3: Xaa = R or V or K or S or N or I or Y
  VARIANT 4: Xaa = V or N or I or R or S or T
  VARIANT 5: Xaa = R or K or I or N
  VARIANT 6: Xaa = G or I or R or K or S or A
XXXXXX

SEQ ID NO: 186 - protein, 8 aa, Artificial Sequence
  Synthetic Construct
  VARIANT 1: Xaa = A or R or M or V or G or S
  VARIANT 2: Xaa = N or T or S or A
  VARIANT 3: Xaa = R or N or H
  VARIANT 4: Xaa = V or R or K
  VARIANT 5: Xaa = K or V or I
  VARIANT 6: Xaa = R or K or A or N or S or V
  VARIANT 7: Xaa = T or G or R or K or P
  VARIANT 8: Xaa = S or G or R or A
XXXXXXXX

SEQ ID NO: 187 - protein, 10 aa, Artificial Sequence
  Synthetic Construct
  VARIANT 1: Xaa = R or A or Q
  VARIANT 2: Xaa = S or A
  VARIANT 3: Xaa = G or S or N or I
  VARIANT 4: Xaa = N or K
  VARIANT 5: Xaa = T or S or L or R
  VARIANT 6: Xaa = I or R or V
  VARIANT 7: Xaa = R or E or K
  VARIANT 8: Xaa = K or Q or A or R
  VARIANT 9: Xaa = R or G or Q
  VARIANT 10: Xaa = E or W or G or R
XXXXXXXXXX

SEQ ID NO: 188 - protein, 5 aa, Artificial Sequence
  Synthetic Construct
  VARIANT 1: Xaa = G or S or N or Y or A or R
  VARIANT 2: Xaa = P or G or S or V or E or R or F or D
  VARIANT 3: Xaa = N or G or S or E or P or K or H or R
  VARIANT 4: Xaa = G or R or H or S or Q or V or D
  VARIANT 5: Xaa = F or D or N or R or G or Y or S or T
XXXXX

SEQ ID NO: 189 - protein, 30 aa, Artificial Sequence
  Synthetic Construct
GCRTNRVKGGCKQDSDCLAGCVCGPNGFCG

SEQ ID NO: 190 - protein, 28 aa, Artificial Sequence
  Synthetic Construct
GCVNRVRGCKQDSDCLAGCVCSGGRDCG

SEQ ID NO: 191 - protein, 30 aa, Artificial Sequence
  Synthetic Construct
GCMNHVKARRCKQDSDCLAGCVCGPNGFCG

SEQ ID NO: 192 - protein, 28 aa, Artificial Sequence
  Synthetic Construct
GCRSVNKICKQDSDCLAGCVCGSSRNCG

SEQ ID NO: 193 - protein, 28 aa, Artificial Sequence
  Synthetic Construct
GCVNKIKGCKQDSDCLAGCVCGVEGRCG

SEQ ID NO: 194 - protein, 28 aa, Artificial Sequence
  Synthetic Construct
GCRNSIKRCKQNSDCLAGCVCSVGHGCG

SEQ ID NO: 195 - protein, 30 aa, Artificial Sequence
  Synthetic Construct
GCVSNRVNKGCKQDSDCLAGCVCGPNGFCG

SEQ ID NO: 196 - protein, 28 aa, Artificial Sequence
  Synthetic Construct
GCRGNIIKCKQDSDCLAGCVCNESRGCG

SEQ ID NO: 197 - protein, 32 aa, Artificial Sequence
  Synthetic Construct
GCRSGNTIRKRECKQDSDCLAGCVCGGPGGCG

SEQ ID NO: 198 - protein, 32 aa, Artificial Sequence
  Synthetic Construct
GCASSNSIRQGWCKQDSDCLAGCVCGPKSNCG

SEQ ID NO: 199 - protein, 28 aa, Artificial Sequence
  Synthetic Construct
GCRSNRIRCKQDSDCLAGCVCYGHGDCG

SEQ ID NO: 200 - protein, 32 aa, Artificial Sequence
  Synthetic Construct
GCRSNKLREARGCKQDSDCLAGCVCGSRQDCG

SEQ ID NO: 201 - protein, 28 aa, Artificial Sequence
  Synthetic Construct
GCVNSVKRCKQDSDCLAGCVCSRGVNCG

SEQ ID NO: 202 - protein, 30 aa, Artificial Sequence
  Synthetic Construct
GCGSNKIRPRCKQDSDCLAGCVCGPNDFCG

SEQ ID NO: 203 - protein, 28 aa, Artificial Sequence
  Synthetic Construct
GCNRIRNSCKQDSDCLAGCVCGRGDYCG

SEQ ID NO: 204 - protein, 28 aa, Artificial Sequence
  Synthetic Construct
GCSRNSIKCKQDSDCLAGCVCASGSSCG

SEQ ID NO: 205 - protein, 28 aa, Artificial Sequence
  Synthetic Construct
GCSNYVKRCKQDSDCLAGCVCSPGGRCG

SEQ ID NO: 206 - protein, 30 aa, Artificial Sequence
  Synthetic Construct
GCRANRVSGRCKQDSDCLAGCVCGPNGFCG

SEQ ID NO: 207 - protein, 30 aa, Artificial Sequence
  Synthetic Construct
GCSNRVKVRACKQDSDCLAGCVCGPNGFCG

SEQ ID NO: 208 - protein, 28 aa, Artificial Sequence
  Synthetic Construct
GCENRTKGCKQDSDCLAGCVCGFRGTCG

SEQ ID NO: 209 - protein, 28 aa, Artificial Sequence
  Synthetic Construct
GCGNKIRACKQDSDCLAGCVCRDRVGCG

SEQ ID NO: 210 - protein, 30 aa, Artificial Sequence
  Synthetic Construct
GCANRVKRTSCKQDSDCLAGCVCGPNGFCG

SEQ ID NO: 211 - protein, 5 aa, Artificial Sequence
  Synthetic Construct
GESLS

SEQ ID NO: 212 - protein, 8 aa, Artificial Sequence
  Synthetic Construct
  VARIANT 6: Xaa = 3,4-difluoro-L-phenylalanine, 3,4-dichloro-L-phenylalanine, 4-chloro-L-phenylalanine, 3-F,4-Cl-L-phenylalanine, 2-pyridone(NH para)-L-alanine, pyridone(NH meta)-L-alanine, or sulfotyrosine
NIMLPXWG

SEQ ID NO: 213 - protein, 8 aa, Artificial Sequence
  Synthetic Construct
  VARIANT 7: Xaa = 1-Naphthyl alanine, 2-Naphthyl alanine, or 2-chloroindole
NIMLPFXG

SEQ ID NO: 214 - protein, 8 aa, Artificial Sequence
  Synthetic Construct
  VARIANT 3: Xaa = norleucine
DVXQPYWG

SEQ ID NO: 215 - protein, 30 aa, Artificial Sequence
  Synthetic Construct
GCNIMLPYWGCGQSFECLAGCVCQYYQSCG

SEQ ID NO: 216 - protein, 30 aa, Artificial Sequence
  Synthetic Construct
  VARIANT 30: glycine can be capped with C(=O)-oxetane-3yl
GCNIMLPYWGCGRDFECLAGCVCQYYQSCG

SEQ ID NO: 217 - protein, 28 aa, Artificial Sequence
  Synthetic Construct
CNIMLPYWGCGRDFECLAGCVCQYYQSC

SEQ ID NO: 218 - protein, 30 aa, Artificial Sequence
  Synthetic Construct
  VARIANT 5: Xaa = norleucine
GCNIXLPFWGCGRDFECLAGCVCQYYQSCG

SEQ ID NO: 219 - protein, 30 aa, Artificial Sequence
  Synthetic Construct
  VARIANT 9: Xaa = 1-naphthylalanine, or 2-naphthylalanine
GCNIMLPFXGCGRDFECLAGCVCQYYQSCG

SEQ ID NO: 220 - protein, 5 aa, Artificial Sequence
  Synthetic Construct
  VARIANT 3: Xaa = 3-fluorotyrosine, or 4-fluorophenylalanine
QYXQS

SEQ ID NO: 221 - protein, 30 aa, Artificial Sequence
  Synthetic Construct
  VARIANT 1: Xaa = PEG6-propargylglycine
XCNIMLPFWGCGRDFECLAGCVCQYYQSCG

SEQ ID NO: 222 - protein, 30 aa, Artificial Sequence
  Synthetic Construct
GCNIMLPYWGCGRDFECMNQCICQYYQSCG

SEQ ID NO: 223 - protein, 30 aa, Artificial Sequence
  Synthetic Construct
GCNIMLPYWGCGRDFECFYECICQYYQSCG

SEQ ID NO: 224 - protein, 30 aa, Artificial Sequence
  Synthetic Construct
  VARIANT 5: Xaa = norleucine
GCDVXQPYWGCGPDIDCLSNCICHWYNSCG

SEQ ID NO: 225 - protein, 10 aa, Artificial Sequence
  Synthetic Construct
ETDWYPHQID

SEQ ID NO: 226 - protein, 10 aa, Artificial Sequence
  Synthetic Construct
GETVFEQFLW

SEQ ID NO: 227 - protein, 6 aa, Artificial Sequence
  Synthetic Construct
HMMYDY

SEQ ID NO: 228 - protein, 8 aa, Artificial Sequence
  Synthetic Construct
KKWQWWYM

SEQ ID NO: 229 - protein, 10 aa, Artificial Sequence
  Synthetic Construct
PAIQNWKEHP

SEQ ID NO: 230 - protein, 8 aa, Artificial Sequence
  Synthetic Construct
QLMHPFWG

SEQ ID NO: 231 - protein, 6 aa, Artificial Sequence
  Synthetic Construct
HMMYDY

SEQ ID NO: 232 - protein, 10 aa, Artificial Sequence
  Synthetic Construct
  VARIANT 1: Xaa = E or G or P or Q or R or T or V
  VARIANT 2: Xaa = T or E or A or D
  VARIANT 3: Xaa = D or T or I or P
  VARIANT 4: Xaa = W or V or Q or T or W
  VARIANT 5: Xaa = Y or F or N or E or P or K
  VARIANT 6: Xaa = P or E or W or N or P
  VARIANT 7: Xaa = H or Q or K or W or H
  VARIANT 8: Xaa = Q or F or E or A or D or W
  VARIANT 9: Xaa = I or L or H
  VARIANT 10: Xaa = D or W or P or Y or T or M or N
XXXXXXXXXX

SEQ ID NO: 233 - protein, 5 aa, Artificial Sequence
  Synthetic Construct
GPNGF

SEQ ID NO: 234 - protein, 5 aa, Artificial Sequence
  Synthetic Construct
GPNGF

SEQ ID NO: 235 - protein, 5 aa, Artificial Sequence
  Synthetic Construct
EMYDA

SEQ ID NO: 236 - protein, 5 aa, Artificial Sequence
  Synthetic Construct
YPWTE

SEQ ID NO: 237 - protein, 6 aa, Artificial Sequence
  Synthetic Construct
SWWPSL

SEQ ID NO: 238 - protein, 5 aa, Artificial Sequence
  Synthetic Construct
HWYRS

SEQ ID NO: 239 - protein, 32 aa, Artificial Sequence
  Synthetic Construct
GCETDWYPHQIDCKQDSDCLAGCVCGPNGFCG

SEQ ID NO: 240 - protein, 32 aa, Artificial Sequence
  Synthetic Construct
GCGETVFEQFLWCKQDSDCLAGCVCGPNGFCG

SEQ ID NO: 241 - protein, 28 aa, Artificial Sequence
  Synthetic Construct
GCHMMYDYCKQDSDCLAGCVCEMYDACG

SEQ ID NO: 242 - protein, 30 aa, Artificial Sequence
  Synthetic Construct
GCKKWQWWYMCKQDSDCLAGCVCYPWTECG

SEQ ID NO: 243 - protein, 33 aa, Artificial Sequence
  Synthetic Construct
GCPAIQNWKEHPCKQDSDCLAGCVCSWWPSLCG

SEQ ID NO: 244 - protein, 30 aa, Artificial Sequence
  Synthetic Construct
GCQLMHPFWGCKQDSDCLAGCVCHWYRSCG

SEQ ID NO: 245 - protein, 8 aa, Artificial Sequence
  Synthetic Construct
HLFEPLWG

SEQ ID NO: 246 - protein, 8 aa, Artificial Sequence
  Synthetic Construct
QVMRPFWG

SEQ ID NO: 247 - protein, 8 aa, Artificial Sequence
  Synthetic Construct
QVMQPAWG

SEQ ID NO: 248 - protein, 8 aa, Artificial Sequence
  Synthetic Construct
HRLQPLWG

SEQ ID NO: 249 - protein, 8 aa, Artificial Sequence
  Synthetic Construct
ELLQPSWG

SEQ ID NO: 250 - protein, 8 aa, Artificial Sequence
  Synthetic Construct
NVLLPLWG

SEQ ID NO: 251 - protein, 8 aa, Artificial Sequence
  Synthetic Construct
DLMQPLWG

SEQ ID NO: 252 - protein, 8 aa, Artificial Sequence
  Synthetic Construct
NPMLPLWG

SEQ ID NO: 253 - protein, 8 aa, Artificial Sequence
  Synthetic Construct
QVLQPSWG

SEQ ID NO: 254 - protein, 8 aa, Artificial Sequence
  Synthetic Construct
QLLEPMWG

SEQ ID NO: 255 - protein, 8 aa, Artificial Sequence
  Synthetic Construct
KLLQPMWG

SEQ ID NO: 256 - protein, 8 aa, Artificial Sequence
  Synthetic Construct
DRMQPYWG

SEQ ID NO: 257 - protein, 8 aa, Artificial Sequence
  Synthetic Construct
KIMQPLWG

SEQ ID NO: 258 - protein, 8 aa, Artificial Sequence
  Synthetic Construct
NLMHPFWG

SEQ ID NO: 259 - protein, 8 aa, Artificial Sequence
  Synthetic Construct
ALLQPLWG

SEQ ID NO: 260 - protein, 8 aa, Artificial Sequence
  Synthetic Construct
RLLEPSWG

SEQ ID NO: 261 - protein, 8 aa, Artificial Sequence
  Synthetic Construct
HLLLPLWG

SEQ ID NO: 262 - protein, 5 aa, Artificial Sequence
  Synthetic Construct
QWYKS

SEQ ID NO: 263 - protein, 5 aa, Artificial Sequence
  Synthetic Construct
LWYDS

SEQ ID NO: 264 - protein, 5 aa, Artificial Sequence
  Synthetic Construct
QWYQS

SEQ ID NO: 265 - protein, 30 aa, Artificial Sequence
  Synthetic Construct
GCHLFEPLWGCKQDSDCLAGCVCHWYQSCG

SEQ ID NO: 266 - protein, 30 aa, Artificial Sequence
  Synthetic Construct
GCQVMRPFWGCKQDSDCLAGCVCHWYQSCG

SEQ ID NO: 267 - protein, 30 aa, Artificial Sequence
  Synthetic Construct
GCQVMQPAWGCKQDSDCLAGCVCHWYQSCG

SEQ ID NO: 268 - protein, 30 aa, Artificial Sequence
  Synthetic Construct
GCHRLQPLWGCKQDSDCLAGCVCHWYQSCG

SEQ ID NO: 269 - protein, 30 aa, Artificial Sequence
  Synthetic Construct
GCELLQPSWGCKQDSDCLAGCVCHWYQSCG

SEQ ID NO: 270 - protein, 30 aa, Artificial Sequence; identical to SEQ ID NO: 53
  Synthetic Construct

SEQ ID NO: 271 - protein, 30 aa, Artificial Sequence
  Synthetic Construct
GCNVLLPLWGCKQDSDCLAGCVCHWYQSCG

SEQ ID NO: 272 - protein, 30 aa, Artificial Sequence; identical to SEQ ID NO: 56
  Synthetic Construct

SEQ ID NO: 273 - protein, 30 aa, Artificial Sequence
  Synthetic Construct
GCDLMQPLWGCKQDSDCLAGCVCHWYQSCG

SEQ ID NO: 274 - protein, 5 aa, Artificial Sequence
  Synthetic Construct
QMFNS

SEQ ID NO: 275 - protein, 30 aa, Artificial Sequence
  Synthetic Construct
GCQVLQPSWGCKQDSDCLAGCVCHWYQSCG

SEQ ID NO: 276 - protein, 30 aa, Artificial Sequence
  Synthetic Construct
GCQLMQPFWGCKQDSDCLAGCVCRWYNSCG

SEQ ID NO: 277 - protein, 8 aa, Artificial Sequence
  Synthetic Construct
  VARIANT 3: Xaa = norleucine
NIXLPFWG

SEQ ID NO: 278 - protein, 30 aa, Artificial Sequence
  Synthetic Construct
GCQLMQPFWGCKQDSDCLAGCVCRWYHSCG

SEQ ID NO: 279 - protein, 30 aa, Artificial Sequence
  Synthetic Construct
GCQLLEPMWGCKQDSDCLAGCVCHWYNSCG

SEQ ID NO: 280 - protein, 30 aa, Artificial Sequence
  Synthetic Construct
GCKLLQPMWGCKQDSDCLAGCVCRWYQSCG

SEQ ID NO: 281 - protein, 30 aa, Artificial Sequence
  Synthetic Construct
GCDRMQPYWGCKQDSDCLAGCVCQWYKSCG

SEQ ID NO: 282 - protein, 30 aa, Artificial Sequence
  Synthetic Construct
GCKIMQPLWGCKQDSDCLAGCVCLWYDSCG

SEQ ID NO: 283 - protein, 30 aa, Artificial Sequence
  Synthetic Construct
GCNLMHPFWGCKQDSDCLAGCVCHWYQSCG

SEQ ID NO: 284 - protein, 30 aa, Artificial Sequence
  Synthetic Construct
GCALLQPLWGCKQDSDCLAGCVCRWYNSCG

SEQ ID NO: 285 - protein, 30 aa, Artificial Sequence
  Synthetic Construct
GCRLLEPSWGCKQDSDCLAGCVCQWYQSCG

SEQ ID NO: 286 - protein, 30 aa, Artificial Sequence
  Synthetic Construct
GCHLLLPLWGCKQDSDCLAGCVCRWYHSCG

SEQ ID NO: 287 - protein, 10 aa, Artificial Sequence
  Synthetic Construct
DDPSFDWSVY

SEQ ID NO: 288 - protein, 10 aa, Artificial Sequence
  Synthetic Construct
WDPTFNWALY

SEQ ID NO: 289 - protein, 10 aa, Artificial Sequence
  Synthetic Construct
QDPTLNWATY

SEQ ID NO: 290 - protein, 10 aa, Artificial Sequence
  Synthetic Construct
EDPTVDWAQY

SEQ ID NO: 291 - protein, 10 aa, Artificial Sequence
  Synthetic Construct
KDTTFNWGLF

SEQ ID NO: 292 - protein, 5 aa, Artificial Sequence
  Synthetic Construct
RMYDS

SEQ ID NO: 293 - protein, 32 aa, Artificial Sequence
  Synthetic Construct
GCDDPSFDWSVYCKQDSDCLAGCVCRMYDSCG

SEQ ID NO: 294 - protein, 32 aa, Artificial Sequence
  Synthetic Construct
GCWDPTFNWALYCKQDSDCLAGCVCQMYDSCG

SEQ ID NO: 295 - protein, 32 aa, Artificial Sequence
  Synthetic Construct
GCQDPTLNWATYCKQDSDCLAGCVCQMYQSCG

SEQ ID NO: 296 - protein, 32 aa, Artificial Sequence
  Synthetic Construct
GCEDPTVDWAQYCKQDSDCLAGCVCQMYQSCG

SEQ ID NO: 297 - protein, 32 aa, Artificial Sequence
  Synthetic Construct
GCKDTTFNWGLFCKQDSDCLAGCVCQLYQSCG

SEQ ID NO: 298 - protein, 5 aa, Artificial Sequence
  Synthetic Construct
GPELN

SEQ ID NO: 299 - protein, 5 aa, Artificial Sequence
  Synthetic Construct
QADYA

SEQ ID NO: 300 - protein, 5 aa, Artificial Sequence
  Synthetic Construct
GVDYL

SEQ ID NO: 301 - protein, 5 aa, Artificial Sequence
  Synthetic Construct
GTNFL

SEQ ID NO: 302 - protein, 5 aa, Artificial Sequence
  Synthetic Construct
SRDFD

SEQ ID NO: 303 - protein, 5 aa, Artificial Sequence
  Synthetic Construct
NRDFL

SEQ ID NO: 304 - protein, 5 aa, Artificial Sequence
  Synthetic Construct
GWDQF

SEQ ID NO: 305 - protein, 5 aa, Artificial Sequence
  Synthetic Construct
GKDFH

SEQ ID NO: 306 - protein, 5 aa, Artificial Sequence
  Synthetic Construct
SGDFA

SEQ ID NO: 307 - protein, 5 aa, Artificial Sequence
  Synthetic Construct
GKELN

SEQ ID NO: 308 - protein, 5 aa, Artificial Sequence
  Synthetic Construct
GWSMD

SEQ ID NO: 309 - protein, 5 aa, Artificial Sequence
  Synthetic Construct
GYDLQ

SEQ ID NO: 310 - protein, 30 aa, Artificial Sequence
  Synthetic Construct
GCNIMLPFWGCGPELNCLAGCVCQYYQSCG

SEQ ID NO: 311 - protein, 30 aa, Artificial Sequence
  Synthetic Construct
GCNIMLPFWGCQADYACLAGCVCQYYQSCG

SEQ ID NO: 312 - protein, 30 aa, Artificial Sequence
  Synthetic Construct
GCNIMLPFWGCGVDYLCLAGCVCQYYQSCG

SEQ ID NO: 313 - protein, 30 aa, Artificial Sequence
  Synthetic Construct
GCNIMLPFWGCGTNFLCLAGCVCQYYQSCG

SEQ ID NO: 314 - protein, 30 aa, Artificial Sequence
  Synthetic Construct
GCNIMLPFWGCSRDFDCLAGCVCQYYQSCG

SEQ ID NO: 315 - protein, 30 aa, Artificial Sequence
  Synthetic Construct
GCNIMLPFWGCNRDFLCLAGCVCQYYQSCG

SEQ ID NO: 316 - protein, 30 aa, Artificial Sequence
  Synthetic Construct
GCNIMLPFWGCGWDQFCLAGCVCQYYQSCG

SEQ ID NO: 317 - protein, 30 aa, Artificial Sequence
  Synthetic Construct
GCNIMLPFWGCGKDFHCLAGCVCQYYQSCG

SEQ ID NO: 318 - protein, 30 aa, Artificial Sequence
  Synthetic Construct
GCNIMLPFWGCSGDFACLAGCVCQYYQSCG

SEQ ID NO: 319 - protein, 30 aa, Artificial Sequence
  Synthetic Construct
GCNIMLPFWGCGKELNCLAGCVCQYYQSCG

SEQ ID NO: 320 - protein, 30 aa, Artificial Sequence
  Synthetic Construct
GCNIMLPFWGCGWSMDCLAGCVCQYYQSCG

SEQ ID NO: 321 - protein, 30 aa, Artificial Sequence
  Synthetic Construct
GCNIMLPFWGCGYDLQCLAGCVCQYYQSCG

SEQ ID NO: 322 - protein, 5 aa, Artificial Sequence
  Synthetic Construct
GRDLQ

SEQ ID NO: 323 - protein, 5 aa, Artificial Sequence
  Synthetic Construct
GVDLS

SEQ ID NO: 324 - protein, 5 aa, Artificial Sequence
  Synthetic Construct
GDDLE

SEQ ID NO: 325 - protein, 5 aa, Artificial Sequence
  Synthetic Construct
GVDMT

SEQ ID NO: 326 - protein, 5 aa, Artificial Sequence
  Synthetic Construct
GMDIE

SEQ ID NO: 327 - protein, 5 aa, Artificial Sequence
  Synthetic Construct
DGDYQ

SEQ ID NO: 328 - protein, 5 aa, Artificial Sequence
  Synthetic Construct
GNDVS

SEQ ID NO: 329 - protein, 5 aa, Artificial Sequence
  Synthetic Construct
AGDEL

SEQ ID NO: 330 - protein, 5 aa, Artificial Sequence
  Synthetic Construct
GLDEE

SEQ ID NO: 331 - protein, 5 aa, Artificial Sequence
  Synthetic Construct
DGDFD

SEQ ID NO: 332 - protein, 5 aa, Artificial Sequence
  Synthetic Construct
AGDFE

SEQ ID NO: 333 - protein, 5 aa, Artificial Sequence
  Synthetic Construct
GNSFE

SEQ ID NO: 334 - protein, 5 aa, Artificial Sequence
  Synthetic Construct
GQDLT

SEQ ID NO: 335 - protein, 5 aa, Artificial Sequence
  Synthetic Construct
GENLA

SEQ ID NO: 336 - protein, 5 aa, Artificial Sequence
  Synthetic Construct
GQDYN

SEQ ID NO: 337 - protein, 5 aa, Artificial Sequence
  Synthetic Construct
GADLS

SEQ ID NO: 338 - protein, 5 aa, Artificial Sequence
  Synthetic Construct
GFDMD

SEQ ID NO: 339 - protein, 5 aa, Artificial Sequence
  Synthetic Construct
DLNYE

SEQ ID NO: 340 - protein, 30 aa, Artificial Sequence
  Synthetic Construct
GCDVMQPYWGCGRDLQCLAGCVCHWYNSCG

SEQ ID NO: 341 - protein, 30 aa, Artificial Sequence
  Synthetic Construct
GCDVMQPYWGCGVDLSCLAGCVCHWYNSCG

SEQ ID NO: 342 - protein, 30 aa, Artificial Sequence
  Synthetic Construct
GCDVMQPYWGCGDDLECLAGCVCHWYNSCG

SEQ ID NO: 343 - protein, 30 aa, Artificial Sequence
  Synthetic Construct
GCDVMQPYWGCGVDMTCLAGCVCHWYNSCG

SEQ ID NO: 344 - protein, 30 aa, Artificial Sequence
  Synthetic Construct
GCDVMQPYWGCGMDIECLAGCVCHWYNSCG

SEQ ID NO: 345 - protein, 30 aa, Artificial Sequence
  Synthetic Construct
GCDVMQPYWGCDGDYQCLAGCVCHWYNSCG

SEQ ID NO: 346 - protein, 30 aa, Artificial Sequence
  Synthetic Construct
GCDVMQPYWGCGNDVSCLAGCVCHWYNSCG

SEQ ID NO: 347 - protein, 30 aa, Artificial Sequence
  Synthetic Construct
GCDVMQPYWGCAGDELCLAGCVCHWYNSCG

SEQ ID NO: 348 - protein, 30 aa, Artificial Sequence
  Synthetic Construct
GCDVMQPYWGCGLDEECLAGCVCHWYNSCG

SEQ ID NO: 349 - protein, 30 aa, Artificial Sequence
  Synthetic Construct
GCDVMQPYWGCDGDFDCLAGCVCHWYNSCG

SEQ ID NO: 350 - protein, 30 aa, Artificial Sequence
  Synthetic Construct
GCDVMQPYWGCAGDFECLAGCVCHWYNSCG

SEQ ID NO: 351 - protein, 30 aa, Artificial Sequence
  Synthetic Construct
GCDVMQPYWGCGNSFECLAGCVCHWYNSCG

SEQ ID NO: 352 - protein, 30 aa, Artificial Sequence
  Synthetic Construct
GCDVMQPYWGCGQDLTCLAGCVCHWYNSCG

SEQ ID NO: 353 - protein, 30 aa, Artificial Sequence
  Synthetic Construct
GCDVMQPYWGCGENLACLAGCVCHWYNSCG

SEQ ID NO: 354 - protein, 30 aa, Artificial Sequence
  Synthetic Construct
GCDVMQPYWGCGQDYNCLAGCVCHWYNSCG

SEQ ID NO: 355 - protein, 30 aa, Artificial Sequence
  Synthetic Construct
GCDVMQPYWGCGADLSCLAGCVCHWYNSCG

SEQ ID NO: 356 - protein, 30 aa, Artificial Sequence
  Synthetic Construct
GCDVMQPYWGCGFDMDCLAGCVCHWYNSCG

SEQ ID NO: 357 - protein, 30 aa, Artificial Sequence
  Synthetic Construct
GCDVMQPYWGCDLNYECLAGCVCHWYNSCG

SEQ ID NO: 358 - protein, 8 aa, Artificial Sequence
  Synthetic Construct
  VARIANT 1: Xaa = Q or H or E or N or D
  VARIANT 2: Xaa = L or V or R or P or I
  VARIANT 3: Xaa = M or F or L
  VARIANT 4: Xaa = Q or E or R or L
  VARIANT 6: Xaa = F or A or L or S
XXXXPXWG

SEQ ID NO: 359 - protein, 5 aa, Artificial Sequence
  Synthetic Construct
  VARIANT 1: Xaa = R or H
  VARIANT 4: Xaa = N or Q or H
XWYXS

SEQ ID NO: 360 - protein, 5 aa, Artificial Sequence
  Synthetic Construct
  VARIANT 1: Xaa = H or L or R or Q
  VARIANT 2: Xaa = W or F or Y
  VARIANT 4: Xaa = Q or N or K or H or D or E
XXYXS

SEQ ID NO: 361 - protein, 30 aa, Artificial Sequence
  Synthetic Construct
  VARIANT 1: Xaa = acetylglycine
XCNIMLPYWGCGRDFECLAGCVCQYYQSCG

SEQ ID NO: 362 - protein, 30 aa, Artificial Sequence
  Synthetic Construct
  VARIANT 8: Xaa = sulfotyrosine, 3,4-difluoro-L-phenylalanine, 3,4-dichloro-L-phenylalanine, 4-chloro-L-phenylalanine, 3-F,4-Cl-L-phenylalanine, 2-pyridone(NH para)-L-alanine, or pyridone(NH meta)-L-alanine
GCNIMLPXWGCGRDFECLAGCVCQYYQSCG

SEQ ID NO: 363 - protein, 30 aa, Artificial Sequence
  Synthetic Construct
GCNIMLPYWGCGRDFECMSDCICQYYQSCG

SEQ ID NO: 364 - protein, 30 aa, Artificial Sequence; identical to SEQ ID NO: 363
  Synthetic Construct

SEQ ID NO: 365 - protein, 30 aa, Artificial Sequence
  Synthetic Construct
  VARIANT 5: Xaa = norleucine
GCNIXLPYWGCGRDFECMSDCICQYYQSCG

SEQ ID NO: 366 - protein, 32 aa, Artificial Sequence
  Synthetic Construct
GCQAINRVKRQRCKQDSDCLAGCVCGPNGFCG

SEQ ID NO: 367 - protein, 10 aa, Artificial Sequence
  Synthetic Construct
QAINRVKRQR

SEQ ID NO: 368 - protein, 8 aa, Artificial Sequence
  Synthetic Construct
NPMLPFWG

SEQ ID NO: 369 - protein, 33 aa, Artificial Sequence
  Synthetic Construct
GCNIMLPFWGCGRDFECLAGCVCQYYQSCGPLI

SEQ ID NO: 370 - protein, 33 aa, Artificial Sequence
  Synthetic Construct
GCNIMLPFWGCGRDFECLAGCVCQYYQSCGNYQ

SEQ ID NO: 371 - protein, 33 aa, Artificial Sequence
  Synthetic Construct
GCNIMLPFWGCGRDFECLAGCVCQYYQSCGPLQ

SEQ ID NO: 372 - protein, 33 aa, Artificial Sequence
  Synthetic Construct
GCNIMLPFWGCGRDFECLAGCVCQYYQSCGTFQ

SEQ ID NO: 373 - protein, 33 aa, Artificial Sequence
  Synthetic Construct
GCNIMLPFWGCGRDFECLAGCVCQYYQSCGDLV

SEQ ID NO: 374 - protein, 33 aa, Artificial Sequence
  Synthetic Construct
GCNIMLPFWGCGRDFECLAGCVCQYYQSCGEHK

SEQ ID NO: 375 - protein, 33 aa, Artificial Sequence
  Synthetic Construct
GCNIMLPFWGCGRDFECLAGCVCQYYQSCGYLS

SEQ ID NO: 376 - protein, 33 aa, Artificial Sequence
  Synthetic Construct
GCNIMLPFWGCGRDFECLAGCVCQYYQSCGWDY

SEQ ID NO: 377 - protein, 33 aa, Artificial Sequence
  Synthetic Construct
GCNIMLPFWGCGRDFECLAGCVCQYYQSCGWPH

SEQ ID NO: 378 - protein, 33 aa, Artificial Sequence
  Synthetic Construct
GCNIMLPFWGCGRDFECLAGCVCQYYQSCGPHQ

SEQ ID NO: 379 - protein, 32 aa, Artificial Sequence
  Synthetic Construct
GCNIMLPFWGCGRDFECLAGCVCQYYQSCGFH

SEQ ID NO: 380 - protein, 32 aa, Artificial Sequence
  Synthetic Construct
GCNIMLPFWGCGRDFECLAGCVCQYYQSCGIA

SEQ ID NO: 381 - protein, 32 aa, Artificial Sequence
  Synthetic Construct
GCNIMLPFWGCGRDFECLAGCVCQYYQSCGGS

SEQ ID NO: 382 - protein, 32 aa, Artificial Sequence
  Synthetic Construct
GCNIMLPFWGCGRDFECLAGCVCQYYQSCGTR

SEQ ID NO: 383 - protein, 32 aa, Artificial Sequence
  Synthetic Construct
GCNIMLPFWGCGRDFECLAGCVCQYYQSCGVH

SEQ ID NO: 384 - protein, 32 aa, Artificial Sequence
  Synthetic Construct
GCNIMLPFWGCGRDFECLAGCVCQYYQSCGLS

SEQ ID NO: 385 - protein, 8 aa, Artificial Sequence
  Synthetic Construct
DVLQPYWG

SEQ ID NO: 386 - protein, 30 aa, Artificial Sequence
  Synthetic Construct
GCDVLQPYWGCGPDIDCLSNCICHWYNSCG

SEQ ID NO: 387 - protein, 32 aa, Artificial Sequence
  Synthetic Construct
GCDVLQPYWGCGPDIDCLSNCICHWYNSCGRT

SEQ ID NO: 388 - protein, 32 aa, Artificial Sequence
  Synthetic Construct
GCDVLQPYWGCGPDIDCLSNCICHWYNSCGWK

SEQ ID NO: 389 - protein, 32 aa, Artificial Sequence
  Synthetic Construct
GCDVLQPYWGCGPDIDCLSNCICHWYNSCGPL

SEQ ID NO: 390 - protein, 32 aa, Artificial Sequence
  Synthetic Construct
GCDVLQPYWGCGPDIDCLSNCICHWYNSCGDE

SEQ ID NO: 391 - protein, 32 aa, Artificial Sequence
  Synthetic Construct
GCDVLQPYWGCGPDIDCLSNCICHWYNSCGQF

SEQ ID NO: 392 - protein, 32 aa, Artificial Sequence
  Synthetic Construct
GCDVLQPYWGCGPDIDCLSNCICHWYNSCGEQ

SEQ ID NO: 393 - protein, 32 aa, Artificial Sequence
  Synthetic Construct
GCDVLQPYWGCGPDIDCLSNCICHWYNSCGPT

SEQ ID NO: 394 - protein, 32 aa, Artificial Sequence
  Synthetic Construct
GCDVLQPYWGCGPDIDCLSNCICHWYNSCGRL

SEQ ID NO: 395 - protein, 32 aa, Artificial Sequence
  Synthetic Construct
GCDVLQPYWGCGPDIDCLSNCICHWYNSCGSL

SEQ ID NO: 396 - protein, 8 aa, Artificial Sequence
  Synthetic Construct
NILLPFWG

SEQ ID NO: 397 - protein, 8 aa, Artificial Sequence
  Synthetic Construct
NILLPYWG

SEQ ID NO: 398 - protein, 8 aa, Artificial Sequence
  Synthetic Construct
NIMSPFWG

SEQ ID NO: 399 - protein, 8 aa, Artificial Sequence
  Synthetic Construct
NIMTPFWG

SEQ ID NO: 400 - protein, 8 aa, Artificial Sequence
  Synthetic Construct
NIMQPFWG

SEQ ID NO: 401 - protein, 8 aa, Artificial Sequence
  Synthetic Construct
NIMNPFWG

SEQ ID NO: 402 - protein, 8 aa, Artificial Sequence
  Synthetic Construct
NIMEPFWG

SEQ ID NO: 403 - protein, 8 aa, Artificial Sequence
  Synthetic Construct
NIMDPFWG

SEQ ID NO: 404 - protein, 8 aa, Artificial Sequence
  Synthetic Construct
  VARIANT 5: Xaa = benzyl-L-proline, 4-fluoro-benzyl-L-proline, 3-OH-L-proline, 3-fluoro-L-proline, or trifluoromethyl-benzyl-L-proline
NIMLXFWG

SEQ ID NO: 405 - protein, 30 aa, Artificial Sequence
  Synthetic Construct
GCNILLPFWGCGRDFECLAGCVCQYYQSCG

SEQ ID NO: 406 - protein, 30 aa, Artificial Sequence
  Synthetic Construct
GCNILLPYWGCGRDFECLAGCVCQYYQSCG

SEQ ID NO: 407 - protein, 30 aa, Artificial Sequence
  Synthetic Construct
GCNIMSPFWGCGRDFECLAGCVCQYYQSCG

SEQ ID NO: 408 - protein, 30 aa, Artificial Sequence
  Synthetic Construct
GCNIMTPFWGCGRDFECLAGCVCQYYQSCG

SEQ ID NO: 409 - protein, 30 aa, Artificial Sequence
  Synthetic Construct
GCNIMQPFWGCGRDFECLAGCVCQYYQSCG

SEQ ID NO: 410 - protein, 30 aa, Artificial Sequence
  Synthetic Construct
GCNIMNPFWGCGRDFECLAGCVCQYYQSCG

SEQ ID NO: 411 - protein, 30 aa, Artificial Sequence
  Synthetic Construct
GCNIMEPFWGCGRDFECLAGCVCQYYQSCG

SEQ ID NO: 412 - protein, 30 aa, Artificial Sequence
  Synthetic Construct
GCNIMDPFWGCGRDFECLAGCVCQYYQSCG

SEQ ID NO: 413 - protein, 30 aa, Artificial Sequence
  Synthetic Construct
  VARIANT 7: Xaa = benzyl-L-proline, 4-fluoro-benzyl-L-proline, 3-OH-L-proline, 3-fluoro-L-proline, or trifluoromethyl-benzyl-L-proline
GCNIMLXFWGCGRDFECLAGCVCQYYQSCG

SEQ ID NO: 414 - protein, 8 aa, Artificial Sequence
  Synthetic Construct
NIMLPSWG

SEQ ID NO: 415 - protein, 30 aa, Artificial Sequence
  Synthetic Construct
GCNIMLPSWGCGRDFECLAGCVCQYYQSCG

SEQ ID NO: 416 - protein, 8 aa, Artificial Sequence
  Synthetic Construct
  VARIANT 7: Xaa = N-methyl indole, N-ethyl indole, N-isopropyl indole, or 5-aza-indole
NIMLPYXG

SEQ ID NO: 417 - protein, 30 aa, Artificial Sequence
  Synthetic Construct
  VARIANT 9: Xaa = N-methyl indole, N-ethyl indole, N-isopropyl indole, or 5-aza-indole
GCNIMLPYXGCGRDFECLAGCVCQYYQSCG

SEQ ID NO: 418 - protein, 5 aa, Artificial Sequence
  Synthetic Construct
  VARIANT 4: Xaa = 4-methyl-L-phenylalanine, 2-naphthyl-L-alanine, 2-quinolyl-Alanine, 4-biphenyl-L-alanine
  VARIANT 4: Xaa = 3-(3-quinolinyl)-L-alanine, 3-(2-quinolinyl)-L-alanine, 3-(2-quinoxalinyl)-L-alanine, 4-methyl-2-pyridyl-alanine
  VARIANT 4: Xaa = 4-ethyl-2-pyridyl-L-alanine, benzothiazole-L-alanine, or benzothiophene-L-alanine, 3-isoquinolinyl-L-alanine
GRDXE

SEQ ID NO: 419 - protein, 30 aa, Artificial Sequence
  Synthetic Construct
  VARIANT 15: Xaa = 4-methyl-L-phenylalanine, 2-naphthyl-L-alanine, 2-quinolyl-Alanine, 4-biphenyl-L-alanine
  VARIANT 15: Xaa = 3-(3-quinolinyl)-L-alanine, 3-(2-quinolinyl)-L-alanine, 3-(2-quinoxalinyl)-L-alanine, 4-methyl-2-pyridyl-alanine
  VARIANT 15: Xaa = 4-ethyl-2-pyridyl-L-alanine, benzothiazole-L-alanine, benzothiophene-L-alanine, or 3-isoquinolinyl-L-alanine
GCNIMLPYWGCGRDXECLAGCVCQYYQSCG

SEQ ID NO: 420 - protein, 30 aa, Artificial Sequence
  Synthetic Construct
  VARIANT 18: Xaa = t-butyl-L-alanine, cyclobutyl-L-alanine, cyclopentyl-L-alanine, or 5,5,5-Trifluoro-L-leucine
GCNIMLPYWGCGRDFECXAGCVCQYYQSCG

SEQ ID NO: 421 - protein, 30 aa, Artificial Sequence
  Synthetic Construct
GCNIMLPFWGCGRDFECLSGCVCQYYQSCG

SEQ ID NO: 422 - protein, 30 aa, Artificial Sequence
  Synthetic Construct
GCNIMLPFWGCGRDFECLTGCVCQYYQSCG

SEQ ID NO: 423 - protein, 30 aa, Artificial Sequence
  Synthetic Construct
GCNIMLPFWGCGRDFECLEGCVCQYYQSCG

SEQ ID NO: 424 - protein, 30 aa, Artificial Sequence
  Synthetic Construct
GCNIMLPYWGCGRDFECLAGCLCQYYQSCG

SEQ ID NO: 425 - protein, 30 aa, Artificial Sequence
  Synthetic Construct
GCNIMLPYWGCGRDFECLAGCICQYYQSCG

SEQ ID NO: 426 - protein, 30 aa, Artificial Sequence
  Synthetic Construct
  VARIANT 22: Xaa = t-butyl-L-glycine (also known as L-tert-Leucine), t-butyl-L-alanine, L-cyclopentylglycine, cyclopentyl-L-alanine
  VARIANT 22: Xaa = L-cyclobutyl-L-glycine, cyclobutyl-L-alanine, or 5,5,5-Trifluoro-L-leucine
GCNIMLPYWGCGRDFECLAGCXCQYYQSCG

SEQ ID NO: 427 - protein, 5 aa, Artificial Sequence
  Synthetic Construct
  VARIANT 2: Xaa = 2-pyridone, 3,4-hydroxy phenylalanine, 3,4-fluoro phenylalanine, or 3-Fluoro,4-OH phenylalanine
QXYQS

SEQ ID NO: 428 - protein, 30 aa, Artificial Sequence
  Synthetic Construct
  VARIANT 25: Xaa = 2-pyridone, 3,4-hydroxy phenylalanine, 3,4-fluoro phenylalanine, or 3-Fluoro,4-OH phenylalanine
GCNIMLPYWGCGRDFECLAGCVCQXYQSCG

SEQ ID NO: 429 - protein, 5 aa, Artificial Sequence
  Synthetic Construct
  VARIANT 3: Xaa = 2-Chloro Tyrosine, 2-Methyl Tyrosine, 2-Ethyl Tyrosine, or 1-naphthol alanine
QYXQS

SEQ ID NO: 430 - protein, 30 aa, Artificial Sequence
  Synthetic Construct
  VARIANT 26: Xaa = 2-Chloro Tyrosine, 2-Methyl Tyrosine, 2-Ethyl Tyrosine, or 1-naphthol alanine
GCNIMLPYWGCGRDFECLAGCVCQYXQSCG

SEQ ID NO: 431 - protein, 30 aa, Artificial Sequence
  Synthetic Construct
GCNIMLPYWGCGRDFECLAGCVCQYYQSCS

SEQ ID NO: 432 - protein, 30 aa, Artificial Sequence
  Synthetic Construct
  VARIANT 30: Xaa = D-serine, L-beta-homoserine, L-beta-alanine, N-alpha-methyl Glycine, glycine amide, glycine ester of glycerol
  VARIANT 30: Xaa = glycine ester of  glycol, glycine ester of oxetane-3-yl alcohol, glycine morpholine amide
GCNIMLPYWGCGRDFECLAGCVCQYYQSCX

SEQ ID NO: 433 - protein, 8 aa, Artificial Sequence
  Synthetic Construct
  VARIANT 3: Xaa = norleucine
NIXQPYWG

SEQ ID NO: 434 - protein, 8 aa, Artificial Sequence
  Synthetic Construct
NILQPYWG

SEQ ID NO: 435 - protein, 30 aa, Artificial Sequence
  Synthetic Construct
GCNILLPYWGCGRDFECMEQCICQYYQSCG

SEQ ID NO: 436 - protein, 30 aa, Artificial Sequence
  Synthetic Construct
  VARIANT 5: Xaa = norleucine
GCNIXQPYWGCGRDFECMEQCICQYYQSCG

SEQ ID NO: 437 - protein, 30 aa, Artificial Sequence
  Synthetic Construct
  VARIANT 5: Xaa = norleucine
  VARIANT 18: Xaa = norleucine or cyclobutyl-L-alanine
GCNIXLPYWGCGRDFECXEQCICQYYQSCG

SEQ ID NO: 438 - protein, 30 aa, Artificial Sequence
  Synthetic Construct
  VARIANT 5: Xaa = norleucine
GCNIXLPYWGCGRDFECLEQCICQYYQSCG

SEQ ID NO: 439 - protein, 30 aa, Artificial Sequence
  Synthetic Construct
  VARIANT 5: Xaa = norleucine
  VARIANT 18: Xaa = cyclobutyl-L-alanine
  VARIANT 22: Xaa = cyclobutyl-L-glycine, cyclobutyl-L-alanine or norleucine
GCNIXLPYWGCGRDFECXEQCXCQYYQSCG

SEQ ID NO: 440 - protein, 30 aa, Artificial Sequence
  Synthetic Construct
  VARIANT 5: Xaa = norleucine
  VARIANT 18: Xaa = cyclobutyl-L-alanine
  VARIANT 22: Xaa = cyclobutyl-L-glycine or cyclobutyl-L-alanine
GCNIXQPYWGCGRDFECXEQCXCQYYQSCG

SEQ ID NO: 441 - protein, 30 aa, Artificial Sequence
  Synthetic Construct
  VARIANT 18: Xaa = cyclobutyl-L-alanine or t-butyl-L-alanine
GCNILLPYWGCGRDFECXEQCICQYYQSCG

SEQ ID NO: 442 - protein, 30 aa, Artificial Sequence
  Synthetic Construct
  VARIANT 22: Xaa = cyclobutyl-L-glycine or cyclobutyl-L-alanine
GCNILLPYWGCGRDFECMEQCXCQYYQSCG

SEQ ID NO: 443 - protein, 30 aa, Artificial Sequence
  Synthetic Construct
  VARIANT 1: Xaa = acetylglycine
  VARIANT 5: Xaa = norleucine
  VARIANT 30: Xaa = glycine amide
XCNIXLPYWGCGRDFECMEQCICQYYQSCX

SEQ ID NO: 444 - protein, 30 aa, Artificial Sequence
  Synthetic Construct
  VARIANT 1: Xaa = acetylglycine
  VARIANT 30: Xaa = glycine amide
XCNILLPYWGCGRDFECMEQCICQYYQSCX

SEQ ID NO: 445 - protein, 30 aa, Artificial Sequence
  Synthetic Construct
  VARIANT 1: Xaa = acetylglycine
  VARIANT 30: Xaa = glycine amide
XCNILQPYWGCGRDFECMEQCICQYYQSCX

SEQ ID NO: 446 - protein, 30 aa, Artificial Sequence
  Synthetic Construct
  VARIANT 1: Xaa = acetylglycine
  VARIANT 30: Xaa = glycine amide
XCNILQPYWGCGRDFECLEQCICQYYQSCX

SEQ ID NO: 447 - protein, 30 aa, Artificial Sequence
  Synthetic Construct
  VARIANT 18: Xaa = cyclobutyl-L-alanine or t-butyl-L-alanine
GCDVLQPYWGCGPDIDCXSNCICHWYNSCG

SEQ ID NO: 448 - protein, 30 aa, Artificial Sequence
  Synthetic Construct
  VARIANT 22: Xaa = cyclobutyl-L-glycine
GCDVLQPYWGCGPDIDCLSNCXCHWYNSCG

SEQ ID NO: 449 - protein, 30 aa, Artificial Sequence
  Synthetic Construct
  VARIANT 5: Xaa = norleucine
  VARIANT 18: Xaa = cyclobutyl-L-alanine
  VARIANT 22: Xaa = cyclobutyl-L-glycine or cyclobutyl-L-alanine
GCDVXQPYWGCGPDIDCXSNCXCHWYNSCG

SEQ ID NO: 450 - protein, 30 aa, Artificial Sequence
  Synthetic Construct
  VARIANT 18: Xaa = cyclobutyl-L-alanine
  VARIANT 22: Xaa = cyclobutyl-L-glycine or cyclobutyl-L-alanine
GCDVLQPYWGCGPDIDCXSNCXCHWYNSCG

SEQ ID NO: 451 - protein, 30 aa, Artificial Sequence
  Synthetic Construct
  VARIANT 1: Xaa = acetylglycine
  VARIANT 18: Xaa = cyclobutyl-L-alanine
  VARIANT 22: Xaa = cyclobutyl-L-glycine or cyclobutyl-L-alanine
  VARIANT 30: Xaa = glycine amide
XCDVLQPYWGCGPDIDCXSNCXCHWYNSCX

SEQ ID NO: 452 - protein, 30 aa, Artificial Sequence
  Synthetic Construct
  VARIANT 1: Xaa = acetylglycine
  VARIANT 5: Xaa = norleucine
  VARIANT 30: Xaa = glycine amide
XCDVXQPYWGCGPDIDCLSNCICHWYNSCX

SEQ ID NO: 453 - protein, 30 aa, Artificial Sequence
  Synthetic Construct
  VARIANT 1: Xaa = acetylglycine
  VARIANT 30: Xaa = glycine amide
XCDVLQPYWGCGPDIDCLSNCICHWYNSCX

SEQ ID NO: 454 - protein, 8 aa, Artificial Sequence
  Synthetic Construct
  VARIANT 3: Xaa = M or L
  VARIANT 4: Xaa = L or S or T or Q or N or E or D
  VARIANT 6: Xaa = F or Y or S
NIXXPXWG

SEQ ID NO: 455 - protein, 32 aa, Artificial Sequence
  Synthetic Construct
GCNIMLPFWGCKQDFDCLAGCICQYYQSCGFH

SEQ ID NO: 456 - protein, 32 aa, Artificial Sequence
  Synthetic Construct
GCDVMQPYWGCEMDFDCLAGCVCHWYNSCGSL

SEQ ID NO: 457 - protein, 32 aa, Artificial Sequence
  Synthetic Construct
GCNIMLPFWGCKQDFDCLAGCICQYYQSCGGE

SEQ ID NO: 458 - protein, 32 aa, Artificial Sequence
  Synthetic Construct
GCNIMLPFWGCKQDSDCLVGCICQYYQSCGSI

SEQ ID NO: 459 - protein, 32 aa, Artificial Sequence
  Synthetic Construct
GCNIMLPFWGCKQDFDCLAGCVCQYYQSCGGR

SEQ ID NO: 460 - protein, 32 aa, Artificial Sequence
  Synthetic Construct
GCNIMLPFWGCKQDFDCLAGCVCQYYQSCGRP

SEQ ID NO: 461 - protein, 32 aa, Artificial Sequence
  Synthetic Construct
GCNIMLPFWGCKQDFDCLAGCVCQYYQSCGQY

SEQ ID NO: 462 - protein, 32 aa, Artificial Sequence
  Synthetic Construct
GCNIMLPFWGCKQDSDCLAGCVCQYYQSCGEN

SEQ ID NO: 463 - protein, 32 aa, Artificial Sequence
  Synthetic Construct
GCNIMLPFWGCKQDFDCLAGCVCQYYQSCGDT

SEQ ID NO: 464 - protein, 32 aa, Artificial Sequence
  Synthetic Construct
GCNIMLPFWGCKQDFDCLAGCVCQYYQSCGQH

SEQ ID NO: 465 - protein, 32 aa, Artificial Sequence
  Synthetic Construct
GCNIMLPFWGCKQDSDCLAGCICQYYQSCGQN

SEQ ID NO: 466 - protein, 32 aa, Artificial Sequence
  Synthetic Construct
GCNIMLPFWGCKQDSDCLAGCVCQYYQSCGEE

SEQ ID NO: 467 - protein, 32 aa, Artificial Sequence
  Synthetic Construct
GCNIMLPFWGCKQDSDCLAGCVCQYYQSCGDD

SEQ ID NO: 468 - protein, 32 aa, Artificial Sequence
  Synthetic Construct
GCNIMLPFWGCKQDSDCLAGCVCQYYQSCGDG

SEQ ID NO: 469 - protein, 32 aa, Artificial Sequence
  Synthetic Construct
GCNIMLPFWGCKQDFDCLAGCVCQYYQSCGLE

SEQ ID NO: 470 - protein, 32 aa, Artificial Sequence
  Synthetic Construct
GCNIMLPFWGCKQDSDCLAGCVCQYYQSCGTD

SEQ ID NO: 471 - protein, 32 aa, Artificial Sequence
  Synthetic Construct
GCNIMLPFWGCKQDSDCLAGCVCQYYQSCGSE

SEQ ID NO: 472 - protein, 32 aa, Artificial Sequence
  Synthetic Construct
GCNIMLPFWGCKQDSDCLAGCVCQYYQSCGPE

SEQ ID NO: 473 - protein, 32 aa, Artificial Sequence
  Synthetic Construct
GCNIMLPFWGCKQDSDCLAGCVCQYYQSCGTN

SEQ ID NO: 474 - protein, 32 aa, Artificial Sequence
  Synthetic Construct
GCNIMLPFWGCKQDSDCLAGCVCQYYQSCGPH

SEQ ID NO: 475 - protein, 32 aa, Artificial Sequence
  Synthetic Construct
GCNIMLPFWGCKQDSDCLAGCVCQYYQSCGMD

SEQ ID NO: 476 - protein, 32 aa, Artificial Sequence
  Synthetic Construct
GCNIMLPFWGCKQDSDCLAGCVCQYYQSCGSD

SEQ ID NO: 477 - protein, 32 aa, Artificial Sequence
  Synthetic Construct
GCNIMLPFWGCGQSFECLAGCICQYYQSCGIA

SEQ ID NO: 478 - protein, 32 aa, Artificial Sequence
  Synthetic Construct
GCNIMLPFWGCGQSFECLAGCICQYYQSCGGS

SEQ ID NO: 479 - protein, 32 aa, Artificial Sequence
  Synthetic Construct
GCNIMLPFWGCGQSFECLAGCICQYYQSCGTR

SEQ ID NO: 480 - protein, 32 aa, Artificial Sequence
  Synthetic Construct
GCNIMLPFWGCGQSFECLAGCICQYYQSCGVH

SEQ ID NO: 481 - protein, 32 aa, Artificial Sequence
  Synthetic Construct
GCDVMQPYWGCKQDFDCLAGCVCHWYNSCGPS

SEQ ID NO: 482 - protein, 32 aa, Artificial Sequence
  Synthetic Construct
GCDVMQPYWGCEMDFDCLAGCICHWYNSCGFS

SEQ ID NO: 483 - protein, 32 aa, Artificial Sequence
  Synthetic Construct
GCDVMQPYWGCEMDFDCLAGCVCHWYNSCGGK

SEQ ID NO: 484 - protein, 32 aa, Artificial Sequence
  Synthetic Construct
GCDVMQPYWGCKQDFDCLAGCICHWYNSCGYL

SEQ ID NO: 485 - protein, 32 aa, Artificial Sequence
  Synthetic Construct
GCDVMQPYWGCEMDFDCLAGCVCHWYNSCGDL

SEQ ID NO: 486 - protein, 32 aa, Artificial Sequence
  Synthetic Construct
GCDVMQPYWGCEMDFDCLAGCVCHWYNSCGEK

SEQ ID NO: 487 - protein, 32 aa, Artificial Sequence
  Synthetic Construct
GCDVMQPYWGCKQDSDCLAGCICHWYNSCGTD

SEQ ID NO: 488 - protein, 32 aa, Artificial Sequence
  Synthetic Construct
GCDVMQPYWGCEMDFDCLAGCICHWYNSCGQV

SEQ ID NO: 489 - protein, 32 aa, Artificial Sequence
  Synthetic Construct
GCDVMQPYWGCEMDFDCLAGCVCHWYNSCGRL

SEQ ID NO: 490 - protein, 32 aa, Artificial Sequence
  Synthetic Construct
GCDVMQPYWGCEMDFDCLAGCICHWYNSCGYA

SEQ ID NO: 491 - protein, 32 aa, Artificial Sequence
  Synthetic Construct
GCDVMQPYWGCEMDFDCLAGCICHWYNSCGAS

SEQ ID NO: 492 - protein, 32 aa, Artificial Sequence
  Synthetic Construct
GCDVMQPYWGCEMDFDCLAGCICHWYNSCGSR

SEQ ID NO: 493 - protein, 32 aa, Artificial Sequence
  Synthetic Construct
GCDVMQPYWGCEMDFDCLAGCICHWYNSCGPT

SEQ ID NO: 494 - protein, 32 aa, Artificial Sequence
  Synthetic Construct
GCDVMQPYWGCEMDFDCLAGCVCHWYNSCGWD

SEQ ID NO: 495 - protein, 32 aa, Artificial Sequence
  Synthetic Construct
GCDVMQPYWGCEMDFDCLAGCVCHWYNSCGSM

SEQ ID NO: 496 - protein, 32 aa, Artificial Sequence
  Synthetic Construct
GCDVMQPYWGCEMDFDCLAGCICHWYNSCGTR

SEQ ID NO: 497 - protein, 32 aa, Artificial Sequence
  Synthetic Construct
GCDVMQPYWGCKQDSDCLAGCVCHWYNSCGEN

SEQ ID NO: 498 - protein, 32 aa, Artificial Sequence
  Synthetic Construct
GCDVMQPYWGCEMDFDCLAGCVCHWYNSCGNN

SEQ ID NO: 499 - protein, 32 aa, Artificial Sequence
  Synthetic Construct
GCDVMQPYWGCEMDFDCLAGCICHWYNSCGPE

SEQ ID NO: 500 - protein, 32 aa, Artificial Sequence
  Synthetic Construct
GCDVMQPYWGCEMDFDCLAGCVCHWYNSCGGI

SEQ ID NO: 501 - protein, 32 aa, Artificial Sequence
  Synthetic Construct
GCDVMQPYWGCEMDFDCLAGCVCHWYNSCGVE

SEQ ID NO: 502 - protein, 32 aa, Artificial Sequence
  Synthetic Construct
GCDVMQPYWGCEMDFDCLAGCVCHWYNSCGPL

SEQ ID NO: 503 - protein, 32 aa, Artificial Sequence; identical to SEQ ID NO: 502
  Synthetic Construct

SEQ ID NO: 504 - protein, 32 aa, Artificial Sequence
  Synthetic Construct
GCDVMQPYWGCEMDFDCLAGCICHWYNSCGRP

SEQ ID NO: 505 - protein, 32 aa, Artificial Sequence
  Synthetic Construct
GCDVMQPYWGCEMDFDCLAGCVCHWYNSCGND

SEQ ID NO: 506 - protein, 32 aa, Artificial Sequence
  Synthetic Construct
GCDVMQPYWGCEMDFDCLAGCICHWYNSCGLQ

SEQ ID NO: 507 - protein, 32 aa, Artificial Sequence
  Synthetic Construct
GCDVMQPYWGCEMDFDCLAGCICHWYNSCGDE

SEQ ID NO: 508 - protein, 32 aa, Artificial Sequence
  Synthetic Construct
GCDVMQPYWGCEMDFDCLAGCICHWYNSCGRT

SEQ ID NO: 509 - protein, 32 aa, Artificial Sequence
  Synthetic Construct
GCDVMQPYWGCEIDFDCLAGCVCHWYNSCGQV

SEQ ID NO: 510 - protein, 32 aa, Artificial Sequence; identical to SEQ ID NO: 500
  Synthetic Construct

SEQ ID NO: 511 - protein, 32 aa, Artificial Sequence
  Synthetic Construct
GCDVMQPYWGCEMDFDCLAGCVCHWYNSCGYM

SEQ ID NO: 512 - protein, 32 aa, Artificial Sequence
  Synthetic Construct
GCDVMQPYWGCEMDFDCLAGCVCHWYNSCGGQ

SEQ ID NO: 513 - protein, 32 aa, Artificial Sequence
  Synthetic Construct
GCDVMQPYWGCEMDFDCLAGCVCHWYNSCGTP

SEQ ID NO: 514 - protein, 32 aa, Artificial Sequence
  Synthetic Construct
GCDVMQPYWGCEMDFDCLAGCVCHWYNSCGVN

SEQ ID NO: 515 - protein, 32 aa, Artificial Sequence
  Synthetic Construct
GCDVMQPYWGCEMDFDCLAGCVCHWYNSCGFN

SEQ ID NO: 516 - protein, 32 aa, Artificial Sequence
  Synthetic Construct
GCDVMQPYWGCEMDFDCLAGCVCHWYNSCGEP

SEQ ID NO: 517 - protein, 32 aa, Artificial Sequence
  Synthetic Construct
GCDVMQPYWGCEMDFDCLAGCVCHWYNSCGNS

SEQ ID NO: 518 - protein, 32 aa, Artificial Sequence
  Synthetic Construct
GCDVMQPYWGCEMDFDCLAGCVCHWYNSCGST

SEQ ID NO: 519 - protein, 32 aa, Artificial Sequence
  Synthetic Construct
GCDVMQPYWGCEMDFDCLAGCVCHWYNSCGRY

SEQ ID NO: 520 - protein, 32 aa, Artificial Sequence; identical to SEQ ID NO: 482
  Synthetic Construct

SEQ ID NO: 521 - protein, 32 aa, Artificial Sequence; identical to SEQ ID NO: 488
  Synthetic Construct

SEQ ID NO: 522 - protein, 32 aa, Artificial Sequence; identical to SEQ ID NO: 490
  Synthetic Construct

SEQ ID NO: 523 - protein, 32 aa, Artificial Sequence; identical to SEQ ID NO: 492
  Synthetic Construct

SEQ ID NO: 524 - protein, 32 aa, Artificial Sequence; identical to SEQ ID NO: 493
  Synthetic Construct

SEQ ID NO: 525 - protein, 32 aa, Artificial Sequence; identical to SEQ ID NO: 495
  Synthetic Construct

SEQ ID NO: 526 - protein, 32 aa, Artificial Sequence; identical to SEQ ID NO: 500
  Synthetic Construct

SEQ ID NO: 527 - protein, 32 aa, Artificial Sequence
  Synthetic Construct
GCDVMQPYWGCEMDFDCLAGCICHWYNSCGTS

SEQ ID NO: 528 - protein, 32 aa, Artificial Sequence; identical to SEQ ID NO: 506
  Synthetic Construct

SEQ ID NO: 529 - protein, 32 aa, Artificial Sequence
  Synthetic Construct
GCDVMQPYWGCEMDFDCLVGCVCHWYNSCGDE

SEQ ID NO: 530 - protein, 32 aa, Artificial Sequence; identical to SEQ ID NO: 485
  Synthetic Construct

SEQ ID NO: 531 - protein, 32 aa, Artificial Sequence
  Synthetic Construct
GCDVMQPYWGCEMDFDCLAGCVCHWYNSCGQF

SEQ ID NO: 532 - protein, 32 aa, Artificial Sequence
  Synthetic Construct
GCDVMQPYWGCEMDFDCLAGCICHWYNSCGWK

SEQ ID NO: 533 - protein, 32 aa, Artificial Sequence
  Synthetic Construct
GCNIMLPFWGCGQSFECLAGCICQYYQSCGLS

SEQ ID NO: 534 - protein, 30 aa, Artificial Sequence
  Synthetic Construct
  VARIANT 5: Xaa = norleucine
  VARIANT 16: Xaa = D or E
  VARIANT 20: Xaa = N, K, or ornithine
GCDVXQPYWGCGPDIXCLSXCICHWYNSCG

SEQ ID NO: 535 - protein, 30 aa, Artificial Sequence; identical to SEQ ID NO: 534
  Synthetic Construct
  VARIANT 5: Xaa = norleucine
  VARIANT 16: Xaa = N, K, or ornithine
  VARIANT 20: Xaa = D or E

SEQ ID NO: 536 - protein, 30 aa, Artificial Sequence
  Synthetic Construct
  VARIANT 5: Xaa = norleucine
GCDVXQPYWGCGPDIDCLSKCICHWYNSCG

SEQ ID NO: 537 - protein, 30 aa, Artificial Sequence
  Synthetic Construct
  VARIANT 5: Xaa = norleucine
  VARIANT 20: Xaa = ornithine
GCDVXQPYWGCGPDIDCLSXCICHWYNSCG

SEQ ID NO: 538 - protein, 30 aa, Artificial Sequence
  Synthetic Construct
  VARIANT 5: Xaa = norleucine
  VARIANT 16: Xaa = D or E
  VARIANT 20: Xaa = N, K, or ornithine
GCNIXLPYWGCGRDFXCMEXCICQYYQSCG

SEQ ID NO: 539 - protein, 30 aa, Artificial Sequence; identical to SEQ ID NO: 538
  Synthetic Construct
  VARIANT 5: Xaa = norleucine
  VARIANT 16: Xaa = N or K or ornithine
  VARIANT 20: Xaa = D or E

SEQ ID NO: 540 - protein, 30 aa, Artificial Sequence
  Synthetic Construct
  VARIANT 5: Xaa = norleucine
  VARIANT 16: Xaa = D or E
  VARIANT 20: Xaa = N or K or ornithine
GCNIXLPFWGCGRDFXCVSXCICQYYQSCG

SEQ ID NO: 541 - protein, 30 aa, Artificial Sequence; identical to SEQ ID NO: 540
  Synthetic Construct
  VARIANT 5: Xaa = norleucine
  VARIANT 16: Xaa = N or K or ornithine
  VARIANT 20: Xaa = D or E

SEQ ID NO: 542 - protein, 30 aa, Artificial Sequence
  Synthetic Construct
GCNIMLPYWGCGRDFECLAKCVCQYYQSCG

SEQ ID NO: 543 - protein, 30 aa, Artificial Sequence
  Synthetic Construct
  VARIANT 5: Xaa = norleucine
GCNIXLPYWGCGRDFECMEKCICQYYQSCG

SEQ ID NO: 544 - protein, 30 aa, Artificial Sequence
  Synthetic Construct
  VARIANT 5: Xaa = norleucine
  VARIANT 20: Xaa = ornithine
GCNIXLPYWGCGRDFECMEXCICQYYQSCG

SEQ ID NO: 545 - protein, 30 aa, Artificial Sequence
  Synthetic Construct
  VARIANT 5: Xaa = norleucine
GCNIXLPFWGCGRDFECVSKCICQYYQSCG

SEQ ID NO: 546 - protein, 30 aa, Artificial Sequence
  Synthetic Construct
  VARIANT 5: Xaa = norleucine
  VARIANT 20: Xaa = ornithine
GCNIXLPFWGCGRDFECVSXCICQYYQSCG

SEQ ID NO: 547 - protein, 30 aa, Artificial Sequence
  Synthetic Construct
GCNILLPFWGCGRDFECVSQCICQYYQSCG

SEQ ID NO: 548 - protein, 30 aa, Artificial Sequence
  Synthetic Construct
GCNILQPFWGCGRDFECVSQCICQYYQSCG

SEQ ID NO: 549 - protein, 30 aa, Artificial Sequence
  Synthetic Construct
  VARIANT 5: Xaa = norleucine
  VARIANT 20: Xaa = D or E
GCDVXQPYWGCGPDIKCLSXCICHWYNSCG

SEQ ID NO: 550 - protein, 30 aa, Artificial Sequence
  Synthetic Construct
  VARIANT 5: Xaa = norleucine
GCDVXQPYWGCGPDIKCLSDCICHWYNSCG

SEQ ID NO: 551 - protein, 30 aa, Artificial Sequence
  Synthetic Construct
  VARIANT 5: Xaa = norleucine
GCDVXQPYWGCGPDIKCLSECICHWYNSCG

SEQ ID NO: 552 - protein, 30 aa, Artificial Sequence; identical to SEQ ID NO: 534
  Synthetic Construct
  VARIANT 5: Xaa = norleucine
  VARIANT 16: Xaa = ornithine
  VARIANT 20: Xaa = D or E

SEQ ID NO: 553 - protein, 30 aa, Artificial Sequence
  Synthetic Construct
  VARIANT 5: Xaa = norleucine
  VARIANT 16: Xaa = ornithine
GCDVXQPYWGCGPDIXCLSDCICHWYNSCG

SEQ ID NO: 554 - protein, 30 aa, Artificial Sequence
  Synthetic Construct
  VARIANT 5: Xaa = norleucine
  VARIANT 16: Xaa = ornithine
GCDVXQPYWGCGPDIXCLSECICHWYNSCG

SEQ ID NO: 555 - protein, 30 aa, Artificial Sequence
  Synthetic Construct
  VARIANT 5: Xaa = norleucine
  VARIANT 20: Xaa = D or E
GCNIXLPYWGCGRDFKCMEXCICQYYQSCG

SEQ ID NO: 556 - protein, 30 aa, Artificial Sequence
  Synthetic Construct
  VARIANT 5: Xaa = norleucine
GCNIXLPYWGCGRDFKCMEDCICQYYQSCG

SEQ ID NO: 557 - protein, 30 aa, Artificial Sequence
  Synthetic Construct
  VARIANT 5: Xaa = norleucine
GCNIXLPYWGCGRDFKCMEECICQYYQSCG

SEQ ID NO: 558 - protein, 30 aa, Artificial Sequence; identical to SEQ ID NO: 538
  Synthetic Construct
  VARIANT 5: Xaa = norleucine
  VARIANT 16: Xaa = ornithine
  VARIANT 20: Xaa = D or E

SEQ ID NO: 559 - protein, 30 aa, Artificial Sequence
  Synthetic Construct
  VARIANT 5: Xaa = norleucine
  VARIANT 16: Xaa = ornithine
GCNIXLPYWGCGRDFXCMEDCICQYYQSCG

SEQ ID NO: 560 - protein, 30 aa, Artificial Sequence
  Synthetic Construct
  VARIANT 5, 16: Xaa = norleucine
  VARIANT 16: Xaa = ornithine
GCNIXLPYWGCGRDFXCMEECICQYYQSCG

SEQ ID NO: 561 - protein, 30 aa, Artificial Sequence
  Synthetic Construct
  VARIANT 5: Xaa = norleucine
  VARIANT 20: Xaa = D or E
GCNIXLPFWGCGRDFKCVSXCICQYYQSCG

SEQ ID NO: 562 - protein, 29 aa, Artificial Sequence
  Synthetic Construct
  VARIANT 4: Xaa = norleucine
CNIXLPFWGCGRDFKCVSDCICQYYQSCG

SEQ ID NO: 563 - protein, 29 aa, Artificial Sequence
  Synthetic Construct
  VARIANT 4: Xaa = norleucine
CNIXLPFWGCGRDFKCVSECICQYYQSCG

SEQ ID NO: 564 - protein, 30 aa, Artificial Sequence; identical to SEQ ID NO: 540
  Synthetic Construct
  VARIANT 5: Xaa = norleucine
  VARIANT 16: Xaa = ornithine
  VARIANT 20: Xaa = D or E

SEQ ID NO: 565 - protein, 30 aa, Artificial Sequence
  Synthetic Construct
  VARIANT 5: Xaa = norleucine
  VARIANT 16: Xaa = ornithine
GCNIXLPFWGCGRDFXCVSDCICQYYQSCG

SEQ ID NO: 566 - protein, 30 aa, Artificial Sequence
  Synthetic Construct
  VARIANT 5: Xaa = norleucine
  VARIANT 516: Xaa = ornithine
GCNIXLPFWGCGRDFXCVSECICQYYQSCG

SEQ ID NO: 567 - protein, 5 aa, Artificial Sequence
  Synthetic Construct
RWYES

SEQ ID NO: 568 - protein, 30 aa, Artificial Sequence
  Synthetic Construct
  VARIANT 20: Xaa = ornithine
GCNIMLPYWGCGRDFECLAXCVCQYYQSCG